European Patent Specification EP 3 748 000 B1, published June 28, 2023. Title: UNSPECIFIC PEROXYGENASE ENZYME VARIANTS FOR SELECTIVE FATTY ACID EPOXIDATION OR HYDROXYLATION. Applicant: Consejo Superior de Investigaciones Científicas (CSIC). The sequence listing filed with the application follows.

SEQUENCE LISTING (9 sequences)

SEQ ID NO: 1 - protein, 236 aa, Artificial Sequence
  Recombinant Marasmius rotula unspecific peroxygenase enzyme, rMroUPO
SAHPWKAPGPNDSRGPCPGLNTLANHGFLPRNGRNISVPMIVKAGFEGYNVQSDILILAGKIGMLTSREADTISLEDLKLHGTIEHDASLSREDVAIGDNLHFNEAIFTTLANSNPGADVYNISSAAQVQHDRLADSLARNPNVTNTDLTATIRSSESAFFLTVMSAGDPLRGEAPKKFVNVFFREERMPIKEGWKRSTTPITIPLLGPIIERITELSDWKPTGDNCGAIVLSPEL

SEQ ID NO: 2 - protein, 236 aa, Artificial Sequence
  Variant of the invention which comprises the SEQ ID NO: 1 and the amino acid substitution I153T
SAHPWKAPGPNDSRGPCPGLNTLANHGFLPRNGRNISVPMIVKAGFEGYNVQSDILILAGKIGMLTSREADTISLEDLKLHGTIEHDASLSREDVAIGDNLHFNEAIFTTLANSNPGADVYNISSAAQVQHDRLADSLARNPNVTNTDLTATTRSSESAFFLTVMSAGDPLRGEAPKKFVNVFFREERMPIKEGWKRSTTPITIPLLGPIIERITELSDWKPTGDNCGAIVLSPEL

SEQ ID NO: 3 - protein, 236 aa, Artificial Sequence
  Variant of the invention which comprises the SEQ ID NO: 1 and the amino acid substitutions I153F and S156F
SAHPWKAPGPNDSRGPCPGLNTLANHGFLPRNGRNISVPMIVKAGFEGYNVQSDILILAGKIGMLTSREADTISLEDLKLHGTIEHDASLSREDVAIGDNLHFNEAIFTTLANSNPGADVYNISSAAQVQHDRLADSLARNPNVTNTDLTATFRSFESAFFLTVMSAGDPLRGEAPKKFVNVFFREERMPIKEGWKRSTTPITIPLLGPIIERITELSDWKPTGDNCGAIVLSPEL

SEQ ID NO: 4 - protein, 28 aa, Artificial Sequence
  Signal peptide
MKLAISSSLIALVSVTTALANSQDVVDF

SEQ ID NO: 5 - DNA, 36 bp, Artificial Sequence
  Forward primer for the I153S mutation
ccgatttaactgcgacttcccgctcttcagaatctg

SEQ ID NO: 6 - DNA, 36 bp, Artificial Sequence
  Forward primer for the I153T mutation
ccgatttaactgcgactacccgctcttcagaatctg

SEQ ID NO: 7 - DNA, 36 bp, Artificial Sequence
  Forward primer for the I153V mutation
ccgatttaactgcgactgtccgctcttcagaatctg

SEQ ID NO: 8 - DNA, 38 bp, Artificial Sequence
  Forward primer for the I153F/S156F mutation
ccgatttaactgcgactttccgctctttcgaatctgcg

SEQ ID NO: 9 - DNA, 795 bp, Artificial Sequence
  Polynucleotide sequence that encodes the enzyme shown in SEQ ID NO: 1
atgaaactggcgatctcttccagcctgatcgccctcgtctcggttaccacagctctggctaacagccaagacgtagttgacttctccgcacatccgtggaaagctccgggtccgaacgactctcgcggtccgtgcccaggcctgaacactctggctaaccacggcttcctgccgcgtaatggtcgtaacatctccgtaccgatgattgtgaaagccggcttcgagggttacaacgtccagagcgacatcctgatcctcgccggtaaaatcggtatgctgacgtcgcgtgaagctgataccatatcgttggaagatctgaaactgcacggtaccatcgaacacgatgcatctctgagccgcgaggatgtagcgattggtgataacctgcacttcaacgaggcaattttcaccaccctggctaactccaaccctggtgcagacgtttataacatttctagcgcggctcaggtgcagcatgatcgtctggcagactctctggcgcgcaacccgaacgttactaacaccgatttaactgcgactatccgctcttcagaatctgcgttcttcctgaccgttatgtccgcaggcgatccgctgcgtggtgaagcgccgaagaaattcgtgaacgtcttctttcgtgaagaacgcatgccgattaaagaaggttggaaacgttccaccaccccgatcactattccgcttctgggtccgatcattgagcgcatcacggaattatcggactggaaaccaactggcgataactgcggcgctatcgttctcagcccggaactgtaa